European Patent Application EP 4 729 602 A1, published April 22, 2026. Title: Antioxidant-producing strain. Applicant: UNIVERSITAT POMPEU FABRA. Application EP EP24383134.4, filed October 15, 2024. The sequence listing filed with the application follows.

SEQUENCE LISTING (24 sequences)

SEQ ID NO: 1 - protein, 23 aa, synthetic construct
MFVQIAASLAAASSIALGIPGAA

SEQ ID NO: 2 - protein, 155 aa, synthetic construct
MEQEVPMNLVSADGKEVSIGKITIQETPYGLLFTPALHSLSEGIHGFHVHEKGNCAPALKDGKPVAALSAGGHFDPKNTGKHLGPWSPDGHLGDLPALFVTHDGKANYPVLAPRLNSLKEIKGRSLMLHAGGDNHHDHPEPLGGGGARMACGIIQ

SEQ ID NO: 3 - DNA, 180 bp, synthetic construct
  source 1..180: mol_type = other DNA
acaccgacgatctgcacgggcgagtctaggggttatcggctacatgcgcgtcgccgcatcaggttcacgaaaccgaaaggcagacccaccccctaccgggcataccgttgccgccgacacttcgatgacactatgcagtgctacacttcaactgaaaatctatatgattttcgtcaattc

SEQ ID NO: 4 - DNA, 69 bp, synthetic construct
  source 1..69: mol_type = other DNA
atgttcgtccaaatcgctgccagcctggcagccgcatcgtccattgcactcggcataccaggagctgcc

SEQ ID NO: 5 - DNA, 194 bp, synthetic construct
  source 1..194: mol_type = other DNA
ggttgatctgtagtgctgccggggccgtgggttccggcagcactgtggactacgggcgggacgcgtgccctctgtgtgagttactgccggtgccctttagctcctttcaatttggggagacgacgttgagaaggtatcgttaactgctggcttcgtgtgtgcggagccacaaccacgcccgcagggggtgtggg

SEQ ID NO: 6 - DNA, 194 bp, synthetic construct
  source 1..194: mol_type = other DNA
cctgtcctgatcatgatccgtccgggggccgctagttgggcggtccccggacgattttgtgtacccgcagatgcgtgccagacaagcgcctcggctgttttgtgggtttgtgttggtggtgggggtgtgtgtagtgtgtgttgggccgttgggggctgcgtgtgtggttcttggtggtggctgtgtttgggatg

SEQ ID NO: 7 - DNA, 29 bp, synthetic construct
  source 1..29: mol_type = other DNA
tccacttataaatatagaggaggtttgat

SEQ ID NO: 8 - DNA, 34 bp, synthetic construct
  source 1..34: mol_type = other DNA
taattttgtttaactttaagaaggagatatacat

SEQ ID NO: 9 - DNA, 489 bp, synthetic construct
  source 1..489: mol_type = other DNA
atggagcaggaagtgccgatgaacctggtctcggctgatggcaaggaggtttccatcgggaagatcaccatccaggagaccccatacggtctgttgttcacccccgccctgcactcgctgagcgagggtattcacggtttccacgtccacgagaagggcaactgcgccccggcgcttaaagacggcaagccggtcgccgcgctgtccgccggtggtcactttgacccgaagaatactggcaagcacctgggcccgtggtcccctgacggccacctcggtgacctgccggccctgttcgtcacccatgacggcaaagccaactacccggtcctggccccgcgcctcaactccctgaaggagatcaagggccgctccctcatgctccacgctggtggcgacaatcaccacgaccacccagagcccctgggcggtggcggtgcccgcatggcctgcggcattatccagcatcatcaccatcaccactgataa

SEQ ID NO: 10 - DNA, 873 bp, synthetic construct
  source 1..873: mol_type = other DNA
cagcctgcggtccggggttgatctgtagtgctgccggggccgtgggttccggcagcactgtggactacgggcgggacgcgtgccctctgtgtgagttactgccggtgccctttagctcctttcaatttggggagacgacgttgagaaggtatcgttaactgctggcttcgtgtgtgcggagccacaaccacgcccgcagggggtgtgggtcgctgggacgcccgtagaactctgtgaggataaagtctcccttacagcctgcggtccggtaattttgtttaactttaagaaggagatatacatatgttcgtccaaatcgctgccagcctggcagccgcatcgtccattgcactcggcataccaggagctgccgagcaggaagtgccgatgaacctggtctcggctgatggcaaggaggtttccatcgggaagatcaccatccaggagaccccatacggtctgttgttcacccccgccctgcactcgctgagcgagggtattcacggtttccacgtccacgagaagggcaactgcgccccggcgcttaaagacggcaagccggtcgccgcgctgtccgccggtggtcactttgacccgaagaatactggcaagcacctgggcccgtggtcccctgacggccacctcggtgacctgccggccctgttcgtcacccatgacggcaaagccaactacccggtcctggccccgcgcctcaactccctgaaggagatcaagggccgctccctcatgctccacgctggtggcgacaatcaccacgaccacccagagcccctgggcggtggcggtgcccgcatggcctgcggcattatccagcatcatcaccatcaccactgataatcgctgggacgcccg

SEQ ID NO: 11 - DNA, 873 bp, synthetic construct
  source 1..873: mol_type = other DNA
cagcctgcggtccggcctgtcctgatcatgatccgtccgggggccgctagttgggcggtccccggacgattttgtgtacccgcagatgcgtgccagacaagcgcctcggctgttttgtgggtttgtgttggtggtgggggtgtgtgtagtgtgtgttgggccgttgggggctgcgtgtgtggttcttggtggtggctgtgtttgggatgtcgctgggacgcccgtagaactctgtgaggataaagtctcccttacagcctgcggtccggtaattttgtttaactttaagaaggagatatacatatgttcgtccaaatcgctgccagcctggcagccgcatcgtccattgcactcggcataccaggagctgccgagcaggaagtgccgatgaacctggtctcggctgatggcaaggaggtttccatcgggaagatcaccatccaggagaccccatacggtctgttgttcacccccgccctgcactcgctgagcgagggtattcacggtttccacgtccacgagaagggcaactgcgccccggcgcttaaagacggcaagccggtcgccgcgctgtccgccggtggtcactttgacccgaagaatactggcaagcacctgggcccgtggtcccctgacggccacctcggtgacctgccggccctgttcgtcacccatgacggcaaagccaactacccggtcctggccccgcgcctcaactccctgaaggagatcaagggccgctccctcatgctccacgctggtggcgacaatcaccacgaccacccagagcccctgggcggtggcggtgcccgcatggcctgcggcattatccagcatcatcaccatcaccactgataatcgctgggacgcccg

SEQ ID NO: 12 - DNA, 9049 bp, synthetic construct
  source 1..9049: mol_type = other DNA
gtgcgtgcgggcgtgagcgtttctacgctgcggcgcaggaaatcagagcttgaggctgccggagcgacggtagacccgtccggttgggtggtgccactgcgtgcactcaaggtcgtttttggggtgtcagatgagacctcgaatgcgaataccagtaaatcctgacctgtgagttgtgaattcataggatagattctggaaactttaccgtccgagctccagcctgcggtccggacaccgacgatctgcacgggcgagtctaggggttatcggctacatgcgcgtcgccgcatcaggttcacgaaaccgaaaggcagacccaccccctaccgggcataccgttgccgccgacacttcgatgacactatgcagtgctacacttcaactgaaaatctatatgattttcgtcaattctccacttataaatatagaggaggtttgatatgttcgtccaaatcgctgccagcctggcagccgcatcgtccattgcactcggcataccaggagctgccgagcaggaagtgccgatgaacctggtctcggctgatggcaaggaggtttccatcgggaagatcaccatccaggagaccccatacggtctgttgttcacccccgccctgcactcgctgagcgagggtattcacggtttccacgtccacgagaagggcaactgcgccccggcgcttaaagacggcaagccggtcgccgcgctgtccgccggtggtcactttgacccgaagaatactggcaagcacctgggcccgtggtcccctgacggccacctcggtgacctgccggccctgttcgtcacccatgacggcaaagccaactacccggtcctggccccgcgcctcaactccctgaaggagatcaagggccgctccctcatgctccacgctggtggcgacaatcaccacgaccacccagagcccctgggcggtggcggtgcccgcatggcctgcggcattatccagcatcatcaccatcaccactgataatcgctgggacgcccgctcgagcaataaacagttgatagggcttctccgttaccatggttcagccaaaaaacttaagaccgccggtcttgtccactaccttgcagtaatgcggtggacaggatcggcggttttcttttctcttctcaagctagcgaaatccctgaaactgagactgtagaaaataagcttccgaaactgaacctgttattttacgctacggacgcccggtcatgacgctgagttagtggcgcagctgcgctctgagaacgagtttttacggcgtcaggtcgagcagcaggcgcgcacgatcgaacggcaggctgaggcacacgcggtggtctcagcgcagctcacacgggttggccagcttgaggccggcgacgcagcagcaccgacactggcacccgttgaaaggccggctccgcgacggcggtggtggcagcgtcggtagcggtcaggatcgctctggcgtgacgagtgtgtctggcagtgcgaacagttgctcgaccagtggcagcagaagcgagatcgctgcgtggtgctgttcctcggtcagttcgtcgaggactggcgggtcttgctgcgtccagccgatcgcctcggcggccaaggtcagttccaagctgtgccaacgcacacgcccctcggctgacagctgagtctcgaactgtgcaactggaccggccggaagatgcacgttgccgaggtcgtgagtggccaagcgcacgtcaaagagtgctgcttcgtagccgcgcagaaatggcagtgctcggtcgattcggatcggcctgcccaggtacattccgggccgcttgatgaacgcctccgcgtagaagcgcaccgttctcggcccggcctcgtgatctgtcactgtgcacgctcctctcgatggttctcgacgctaccggagaccaccgacgttcatgcccagcgcagcgacctgaaaggaccaagccgagttagccgtgctaaccgtatagcttgctccgtcgcctctgagggcaaccacctgcgcagcaggtgggcggcagcccgcgcgcaagcgcctaccgggtttgggcacagcccataaatcaacgcctccggtgttgaagcgatcgtgtgtcacgattgctatgcttgctaccccttcagggttttcgtatacacaaatcaagttttttcgtatacgctaatgccatgagtgagcatctactgcacggcaagcccgtcaccaacgagcagattcaggcatgggcagacgaggccgaggccggatacgacctgcccaaactccccaagccacggcgcggacgcccgcccgtaggagacggtccgggcaccgtcgtacccgtgcgtctcgacgcggccaccgttgccgctctcacagaacgagcaacagccgagggcatcacgaaccgttcagacgcgatccgagccgcagtccacgagtggacacgggttgcctgacctccacgactcagcacgcaagcactaccaacgagaccggctcgacgacacggccgtgctctacgcggccacccacgttctcaactcccggccactcgacgacgaagacgacccgcgccgctggctcatgatcggaaccgacccagcaggccgcctactcgaactcgtcgcactgatctacgacgacggctacgaactgatcatccacgcaatgaaagcccgcacccaatacctcgaccagctctaaccaagaaaggaacctgatgagcgaccagctagacagcgaccgcaactacgacccgatgatcttcgacgtgatgcgcgagaccgcgaaccgcgtcgtcgccacgtacgttgcatgggaagatgaagccgctgatccccgcgaggctgcgcactggcaggccgagcgattccgcacccggcacgaggtgcgcgccgtcgaccctgacagccggcgagcagttcaggcgaagatcgcacagctgcgcgaggaactagccgcaatgcccgaacacgccccagccatcccttggagcaggtggcagcgtcaggggagtcgggggatgtttggcaggggatgtggaaagagagttcgctttgctcacatggctcaaccgggtaactaactgatatggggtcttcgtcgcccactttgaacacgccgaggaatggaccacgctgaacgtgactcgcatgcttcactgcatgtatggattcgttcgagacgttgttccctgagagctggctgccacgcaagccgctggcgtcagccgagaagtctggggcgtaccggcacgtgactcggcagagggcgctggagctgccttacatcgaagcgaacccgttggtcatgcagtccttggtcatcaccgatcgagatgcttcggatgctgactgggccgcagacctcgctgggctgccttcaccgtcctacgtgtccatgaaccgtgtcacgaccaccggacacatcgtctatgccttgaagaaccctgtgtgtctgaccgatgccgcgcggcgacggcctatcaacctgctcgcccgcgtcgagcagggcctatgcgacgttctcggcggcgatgcatcctacgggcaccggatcacaaagaacccgctcagcaccgcccatgcgaccctctggggccccgcagacgcgctctacgagctgcgcgccctcgcacacaccctcgacgagatccacgcactgccggaggcagggaacccgcgtcgcaacgtcacccgatcaacggtcggccgcaacgtcaccctgttcgacaccacccgcatgtgggcataccgggccgtccggcactcctggggcggcccggtcgccgaatgggagcacaccgtattcgagcacatccacctactgaacgagacgatcatcgccgacgaattcgccacaggccccctcggcttgaacgaacttaagcacttatctcgatccatttcccgatgggtctggcgcaacttcacccccgaaaccttccgcgcacgccagaaagcgatcagcctccgtggagcatccaaaggcggcaaagaaggcggccacaaaggcggcattgccagtggcgcatcacggcgcgcccatacccgtcaacagttcttggagggtctctcatgaccacacgtgaacgtctcccccgcaacggctacagcatcgccgctgctgcgaaaaagctcggtgtctccgagtccaccgtcaagcggtggacttccgagccacgcgaggagttcgtggcccgcgttgccgcacgccacgcgcggattcgtgagctgcgctcggagggtcagagcatgcgtgcgattgctgccgaggtcggggtttccgtgggcaccgtgcactacgcgctgaacaagaatcgaactgacgcatgaccgtaacgccgcacgatgagcattttcttgatcgtgcaccgcttggcactacgttcgcgtgcggttgcacagtgcgcgccacgttcttatcctgcggccattgtggctacagccaatggggggcatcagcaacggacgttgaacccggtgggcaagtgttactcagggggacatgcccagtctgcggcgctcggattgacggtatggcagtcgtgcatgcggccccaccgtcaaactcattcaggtatcagtgagaaccctcatggcaccccctcgtgacacgttctcgttgcgatcagctgcggccaagcttgatcttcgggcagcgttgggtcctggccacgggtgcgcatgatcgtgctcctgtcgttgaggacccggctaggctggcggggttgccttactggttagcagaatgaatcaccgatacgcgagcgaacgtgaagcgactgctgctgcaaaacgtctgcgacctgagcaacaacatgaatggtcttcggtttccgtgtttcgtaaagtctggaaacgcggaagtcagcgccctgcaccattatgttccggatctgcatcgcaggatgctgctggctaccctgtggaacacctacatctgtattaacgaagcgctggcattgaccctgagtgatttttctctggtcccgccgcatccataccgccagttgtttaccctcacaacgttccagtaaccgggcatgttcatcatcagtaacccgtatcgtgagcatcctctctcgtttcatcggtatcattacccccatgaacagaaatcccccttacacggaggcatcagtgaccaaacaggaaaaaaccgcccttaacatggcccgctttatcagaagccagacattaacgcttctggagaaactcaacgagctggacgcggatgaacaggcagacatctgtgaatcgcttcacgaccacgctgatgagctttaccgcagctgcctcgcgcgtttcggtgatgacggtgaaaacctctgacacatgcagctcccggagacggtcacagcttgtctgtaagcggatgccgggagcagacaagcccgtcagggcgcgtcagcgggtgttggcgggtgtcggggcgcagccatgacccagtcacgtagcgatagcggagtgtatactggcttaactatgcggcatcagagcagattgtactgagagtgcaccatatgcggtgtgaaataccgcacagatgcgtaaggagaaaataccgcatcaggcgctcttccgcttcctcgctcactgactcgctgcgctcggtcgttcggctgcggcgagcggtatcagctcactcaaaggcggtaatacggttatccacagaatcaggggataacgcaggaaagaacatgtgagcaaaaggccagcaaaaggccaggaaccgtaaaaaggccgcgttgctggcgtttttccataggctccgcccccctgacgagcatcacaaaaatcgacgctcaagtcagaggtggcgaaacccgacaggactataaagataccaggcgtttccccctggaagctccctcgtgcgctctcctgttccgaccctgccgcttaccggatacctgtccgcctttctcccttcgggaagcgtggcgctttctcatagctcacgctgtaggtatctcagttcggtgtaggtcgttcgctccaagctgggctgtgtgcacgaaccccccgttcagcccgaccgctgcgccttatccggtaactatcgtcttgagtccaacccggtaagacacgacttatcgccactggcagcagccactggtaacaggattagcagagcgaggtatgtaggcggtgctacagagttcttgaagtggtggcctaactacggctacactagaaggacagtatttggtatctgcgctctgctgaagccagttaccttcggaaaaagagttggtagctcttgatccggcaaacaaaccaccgctggtagcggtggtttttttgtttgcaagcagcagattacgcgcagaaaaaaaggatctcaagaagatcctttgatcttttctacggggtctgacgctcagtggaacgaaaactcacgttaagggattttggtcatgagattatcaaaaaggatcttcacctagatccttttaaattaaaaatgaagttttaaatcaatctaaagtatatatgagtaaacttggtctgacagttaccaatgcttaatcagtgaggcacctatctcagcgatctgtctatttcgttcatccatagttgcctgactccccgtcgtgtagataactacgatacgggagggcttaccatctggccccagtgctgcaatgataccgcgagacccacgctcaccggctccagatttatcagcaataaaccagccagccggaagggccgagcgcagaagtggtcctgcaactttatccgcctccatccagtctattaattgttgccgggaagctagagtaagtagttcgccagttaatagtttgcgcaacgttgttgccattgctgcaggcatcgtggtgtcacgctcgtcgtttggtatggcttcattcagctccggttcccaacgatcaaggcgagttacatgatcccccatgttgtgcaaaaaagcggttagctccttcggtcctccgatcgttgtcagaagtaagttggccgcagtgttatcactcatggttatggcagcactgcataattctcttactgtcatgccatccgtaagatgcttttctgtgactggtgagtactcaaccaagtcattctgagaatagtgtatgcggcgaccgagttgctcttgcccggcgtcaacacgggataataccgcgccacatagcagaactttaaaagtgctcatcattggaaaacgttcttcggggcgaaaactctcaaggatcttaccgctgttgagatccagttcgatgtaacccactcgtgcacccaactgatcttcagcatcttttactttcaccagcgtttctgggtgagcaaaaacaggaaggcaaaatgccgcaaaaaagggaataagggcgacacggaaatgttgaatactcatactcttcctttttcaatattattgaagcatttatcagggttattgtctcatgagcggatacatatttgaatgtatttagaaaaataaacaaataggggttccgcgcacatttccccgaaaagtgccacctgacgtctaagaaaccattattatcatgacattaacctataaaaataggcgtatcacgaggccctttcgtcttcaagaattcaagcttgtcgacgttaacctgcaggcatgcggatccggtaccagctgtctcttatacacatctctgcagttaacgctgacccggaccaccacgacgacccggacgaccaccggtacgaccaccaccagacggaccgcggcgaccaccctggtcaccctgttcacgttcaccggtacgaccgtcgtcacggttacgaccagaagaacgacggtcaccgtgaccagacgcttgccggtctctgcgatcttggcccccggtacgtctgtcaccacggtcctgaccaccggtacgacggtcgcccctatcctgtccacccgtcctacgaccacgctgcggctgaccaccacgcggttcgtttttctggtccagacgttcgaacagacgcagccactgttccggacgaacgtaagcaacaacagcaccaccaccaacaccagcgtggtccagagcagcttcaacacgacgacgcgggtatttacgcagcagagaagcctggatgttaccaccaacaccggtgaagcacagttcaaccatagattcgtaacgttccagagcagcaccttccagcagcggttcagcacgacgacgcagacgcatgatagcagagtcaactttcggaaccggtttgaacagacgacgatcgactttttcaacgaattcccattcgaacagcggccaggtcataacggtcagacgagaccaacgaccgtagtcaccggtacgtttacgagcgaattccagctgggtaaccatggtagcggtttcgatggtcggagcttccaggcaccagtcaacgatagcagaggtgataccgtacgggatagcaccaacgaaagcgaacggttccggcggcggttcagcggtcaggaagtcagcgttaacaacttcgatgttcgggtgaccagacagtttttcacgcagagatttagccagacgcgggtcgatttcgtaagaggtaacctgacgagcacggtcagccagttcacgggtcagcagaccttcacccggaccagcttccagaaccggcaggtccggacgcagttcagcggtttcagcgatacgagcgatggttttacggtcacgcaggaagttctggccgaattggcggcggttacggtcacgctcggtacggccgaggacggggcgattctggttggggtgctggcggtcttggttgcggcggcgggggcggggctgttcatcggaggaggacatgacgatctcccgatgtgtcgtacgtatgggaattgacgaaaatcatatagattttcagttgaagtgtagcactgcatagtgtcatcgaagtgtcggcggcaacggtatgcccggtagggggtgggtctgcctttcggtttcgtgaacctgatgcggcgacgcgcatgtagccgataacccctagactcgcccgtgcagatcgtcggtgtggatccagatgtgtataagagacagctggtaccggccgctgct

SEQ ID NO: 13 - DNA, 9128 bp, synthetic construct
  source 1..9128: mol_type = other DNA
gtgcgtgcgggcgtgagcgtttctacgctgcggcgcaggaaatcagagcttgaggctgccggagcgacggtagacccgtccggttgggtggtgccactgcgtgcactcaaggtcgtttttggggtgtcagatgagacctcgaatgcgaataccagtaaatcctgacctgtgagttgtgaattcataggatagattctggaaactttaccgtccgagctccagcctgcggtccggggttgatctgtagtgctgccggggccgtgggttccggcagcactgtggactacgggcgggacgcgtgccctctgtgtgagttactgccggtgccctttagctcctttcaatttggggagacgacgttgagaaggtatcgttaactgctggcttcgtgtgtgcggagccacaaccacgcccgcagggggtgtgggtcgctgggacgcccgtagaactctgtgaggataaagtctcccttacagcctgcggtccggtaattttgtttaactttaagaaggagatatacatatgttcgtccaaatcgctgccagcctggcagccgcatcgtccattgcactcggcataccaggagctgccgagcaggaagtgccgatgaacctggtctcggctgatggcaaggaggtttccatcgggaagatcaccatccaggagaccccatacggtctgttgttcacccccgccctgcactcgctgagcgagggtattcacggtttccacgtccacgagaagggcaactgcgccccggcgcttaaagacggcaagccggtcgccgcgctgtccgccggtggtcactttgacccgaagaatactggcaagcacctgggcccgtggtcccctgacggccacctcggtgacctgccggccctgttcgtcacccatgacggcaaagccaactacccggtcctggccccgcgcctcaactccctgaaggagatcaagggccgctccctcatgctccacgctggtggcgacaatcaccacgaccacccagagcccctgggcggtggcggtgcccgcatggcctgcggcattatccagcatcatcaccatcaccactgataatcgctgggacgcccgctcgagcaataaacagttgatagggcttctccgttaccatggttcagccaaaaaacttaagaccgccggtcttgtccactaccttgcagtaatgcggtggacaggatcggcggttttcttttctcttctcaagctagcgaaatccctgaaactgagactgtagaaaataagcttccgaaactgaacctgttattttacgctacggacgcccggtcatgacgctgagttagtggcgcagctgcgctctgagaacgagtttttacggcgtcaggtcgagcagcaggcgcgcacgatcgaacggcaggctgaggcacacgcggtggtctcagcgcagctcacacgggttggccagcttgaggccggcgacgcagcagcaccgacactggcacccgttgaaaggccggctccgcgacggcggtggtggcagcgtcggtagcggtcaggatcgctctggcgtgacgagtgtgtctggcagtgcgaacagttgctcgaccagtggcagcagaagcgagatcgctgcgtggtgctgttcctcggtcagttcgtcgaggactggcgggtcttgctgcgtccagccgatcgcctcggcggccaaggtcagttccaagctgtgccaacgcacacgcccctcggctgacagctgagtctcgaactgtgcaactggaccggccggaagatgcacgttgccgaggtcgtgagtggccaagcgcacgtcaaagagtgctgcttcgtagccgcgcagaaatggcagtgctcggtcgattcggatcggcctgcccaggtacattccgggccgcttgatgaacgcctccgcgtagaagcgcaccgttctcggcccggcctcgtgatctgtcactgtgcacgctcctctcgatggttctcgacgctaccggagaccaccgacgttcatgcccagcgcagcgacctgaaaggaccaagccgagttagccgtgctaaccgtatagcttgctccgtcgcctctgagggcaaccacctgcgcagcaggtgggcggcagcccgcgcgcaagcgcctaccgggtttgggcacagcccataaatcaacgcctccggtgttgaagcgatcgtgtgtcacgattgctatgcttgctaccccttcagggttttcgtatacacaaatcaagttttttcgtatacgctaatgccatgagtgagcatctactgcacggcaagcccgtcaccaacgagcagattcaggcatgggcagacgaggccgaggccggatacgacctgcccaaactccccaagccacggcgcggacgcccgcccgtaggagacggtccgggcaccgtcgtacccgtgcgtctcgacgcggccaccgttgccgctctcacagaacgagcaacagccgagggcatcacgaaccgttcagacgcgatccgagccgcagtccacgagtggacacgggttgcctgacctccacgactcagcacgcaagcactaccaacgagaccggctcgacgacacggccgtgctctacgcggccacccacgttctcaactcccggccactcgacgacgaagacgacccgcgccgctggctcatgatcggaaccgacccagcaggccgcctactcgaactcgtcgcactgatctacgacgacggctacgaactgatcatccacgcaatgaaagcccgcacccaatacctcgaccagctctaaccaagaaaggaacctgatgagcgaccagctagacagcgaccgcaactacgacccgatgatcttcgacgtgatgcgcgagaccgcgaaccgcgtcgtcgccacgtacgttgcatgggaagatgaagccgctgatccccgcgaggctgcgcactggcaggccgagcgattccgcacccggcacgaggtgcgcgccgtcgaccctgacagccggcgagcagttcaggcgaagatcgcacagctgcgcgaggaactagccgcaatgcccgaacacgccccagccatcccttggagcaggtggcagcgtcaggggagtcgggggatgtttggcaggggatgtggaaagagagttcgctttgctcacatggctcaaccgggtaactaactgatatggggtcttcgtcgcccactttgaacacgccgaggaatggaccacgctgaacgtgactcgcatgcttcactgcatgtatggattcgttcgagacgttgttccctgagagctggctgccacgcaagccgctggcgtcagccgagaagtctggggcgtaccggcacgtgactcggcagagggcgctggagctgccttacatcgaagcgaacccgttggtcatgcagtccttggtcatcaccgatcgagatgcttcggatgctgactgggccgcagacctcgctgggctgccttcaccgtcctacgtgtccatgaaccgtgtcacgaccaccggacacatcgtctatgccttgaagaaccctgtgtgtctgaccgatgccgcgcggcgacggcctatcaacctgctcgcccgcgtcgagcagggcctatgcgacgttctcggcggcgatgcatcctacgggcaccggatcacaaagaacccgctcagcaccgcccatgcgaccctctggggccccgcagacgcgctctacgagctgcgcgccctcgcacacaccctcgacgagatccacgcactgccggaggcagggaacccgcgtcgcaacgtcacccgatcaacggtcggccgcaacgtcaccctgttcgacaccacccgcatgtgggcataccgggccgtccggcactcctggggcggcccggtcgccgaatgggagcacaccgtattcgagcacatccacctactgaacgagacgatcatcgccgacgaattcgccacaggccccctcggcttgaacgaacttaagcacttatctcgatccatttcccgatgggtctggcgcaacttcacccccgaaaccttccgcgcacgccagaaagcgatcagcctccgtggagcatccaaaggcggcaaagaaggcggccacaaaggcggcattgccagtggcgcatcacggcgcgcccatacccgtcaacagttcttggagggtctctcatgaccacacgtgaacgtctcccccgcaacggctacagcatcgccgctgctgcgaaaaagctcggtgtctccgagtccaccgtcaagcggtggacttccgagccacgcgaggagttcgtggcccgcgttgccgcacgccacgcgcggattcgtgagctgcgctcggagggtcagagcatgcgtgcgattgctgccgaggtcggggtttccgtgggcaccgtgcactacgcgctgaacaagaatcgaactgacgcatgaccgtaacgccgcacgatgagcattttcttgatcgtgcaccgcttggcactacgttcgcgtgcggttgcacagtgcgcgccacgttcttatcctgcggccattgtggctacagccaatggggggcatcagcaacggacgttgaacccggtgggcaagtgttactcagggggacatgcccagtctgcggcgctcggattgacggtatggcagtcgtgcatgcggccccaccgtcaaactcattcaggtatcagtgagaaccctcatggcaccccctcgtgacacgttctcgttgcgatcagctgcggccaagcttgatcttcgggcagcgttgggtcctggccacgggtgcgcatgatcgtgctcctgtcgttgaggacccggctaggctggcggggttgccttactggttagcagaatgaatcaccgatacgcgagcgaacgtgaagcgactgctgctgcaaaacgtctgcgacctgagcaacaacatgaatggtcttcggtttccgtgtttcgtaaagtctggaaacgcggaagtcagcgccctgcaccattatgttccggatctgcatcgcaggatgctgctggctaccctgtggaacacctacatctgtattaacgaagcgctggcattgaccctgagtgatttttctctggtcccgccgcatccataccgccagttgtttaccctcacaacgttccagtaaccgggcatgttcatcatcagtaacccgtatcgtgagcatcctctctcgtttcatcggtatcattacccccatgaacagaaatcccccttacacggaggcatcagtgaccaaacaggaaaaaaccgcccttaacatggcccgctttatcagaagccagacattaacgcttctggagaaactcaacgagctggacgcggatgaacaggcagacatctgtgaatcgcttcacgaccacgctgatgagctttaccgcagctgcctcgcgcgtttcggtgatgacggtgaaaacctctgacacatgcagctcccggagacggtcacagcttgtctgtaagcggatgccgggagcagacaagcccgtcagggcgcgtcagcgggtgttggcgggtgtcggggcgcagccatgacccagtcacgtagcgatagcggagtgtatactggcttaactatgcggcatcagagcagattgtactgagagtgcaccatatgcggtgtgaaataccgcacagatgcgtaaggagaaaataccgcatcaggcgctcttccgcttcctcgctcactgactcgctgcgctcggtcgttcggctgcggcgagcggtatcagctcactcaaaggcggtaatacggttatccacagaatcaggggataacgcaggaaagaacatgtgagcaaaaggccagcaaaaggccaggaaccgtaaaaaggccgcgttgctggcgtttttccataggctccgcccccctgacgagcatcacaaaaatcgacgctcaagtcagaggtggcgaaacccgacaggactataaagataccaggcgtttccccctggaagctccctcgtgcgctctcctgttccgaccctgccgcttaccggatacctgtccgcctttctcccttcgggaagcgtggcgctttctcatagctcacgctgtaggtatctcagttcggtgtaggtcgttcgctccaagctgggctgtgtgcacgaaccccccgttcagcccgaccgctgcgccttatccggtaactatcgtcttgagtccaacccggtaagacacgacttatcgccactggcagcagccactggtaacaggattagcagagcgaggtatgtaggcggtgctacagagttcttgaagtggtggcctaactacggctacactagaaggacagtatttggtatctgcgctctgctgaagccagttaccttcggaaaaagagttggtagctcttgatccggcaaacaaaccaccgctggtagcggtggtttttttgtttgcaagcagcagattacgcgcagaaaaaaaggatctcaagaagatcctttgatcttttctacggggtctgacgctcagtggaacgaaaactcacgttaagggattttggtcatgagattatcaaaaaggatcttcacctagatccttttaaattaaaaatgaagttttaaatcaatctaaagtatatatgagtaaacttggtctgacagttaccaatgcttaatcagtgaggcacctatctcagcgatctgtctatttcgttcatccatagttgcctgactccccgtcgtgtagataactacgatacgggagggcttaccatctggccccagtgctgcaatgataccgcgagacccacgctcaccggctccagatttatcagcaataaaccagccagccggaagggccgagcgcagaagtggtcctgcaactttatccgcctccatccagtctattaattgttgccgggaagctagagtaagtagttcgccagttaatagtttgcgcaacgttgttgccattgctgcaggcatcgtggtgtcacgctcgtcgtttggtatggcttcattcagctccggttcccaacgatcaaggcgagttacatgatcccccatgttgtgcaaaaaagcggttagctccttcggtcctccgatcgttgtcagaagtaagttggccgcagtgttatcactcatggttatggcagcactgcataattctcttactgtcatgccatccgtaagatgcttttctgtgactggtgagtactcaaccaagtcattctgagaatagtgtatgcggcgaccgagttgctcttgcccggcgtcaacacgggataataccgcgccacatagcagaactttaaaagtgctcatcattggaaaacgttcttcggggcgaaaactctcaaggatcttaccgctgttgagatccagttcgatgtaacccactcgtgcacccaactgatcttcagcatcttttactttcaccagcgtttctgggtgagcaaaaacaggaaggcaaaatgccgcaaaaaagggaataagggcgacacggaaatgttgaatactcatactcttcctttttcaatattattgaagcatttatcagggttattgtctcatgagcggatacatatttgaatgtatttagaaaaataaacaaataggggttccgcgcacatttccccgaaaagtgccacctgacgtctaagaaaccattattatcatgacattaacctataaaaataggcgtatcacgaggccctttcgtcttcaagaattcaagcttgtcgacgttaacctgcaggcatgcggatccggtaccagctgtctcttatacacatctctgcagttaacgctgacccggaccaccacgacgacccggacgaccaccggtacgaccaccaccagacggaccgcggcgaccaccctggtcaccctgttcacgttcaccggtacgaccgtcgtcacggttacgaccagaagaacgacggtcaccgtgaccagacgcttgccggtctctgcgatcttggcccccggtacgtctgtcaccacggtcctgaccaccggtacgacggtcgcccctatcctgtccacccgtcctacgaccacgctgcggctgaccaccacgcggttcgtttttctggtccagacgttcgaacagacgcagccactgttccggacgaacgtaagcaacaacagcaccaccaccaacaccagcgtggtccagagcagcttcaacacgacgacgcgggtatttacgcagcagagaagcctggatgttaccaccaacaccggtgaagcacagttcaaccatagattcgtaacgttccagagcagcaccttccagcagcggttcagcacgacgacgcagacgcatgatagcagagtcaactttcggaaccggtttgaacagacgacgatcgactttttcaacgaattcccattcgaacagcggccaggtcataacggtcagacgagaccaacgaccgtagtcaccggtacgtttacgagcgaattccagctgggtaaccatggtagcggtttcgatggtcggagcttccaggcaccagtcaacgatagcagaggtgataccgtacgggatagcaccaacgaaagcgaacggttccggcggcggttcagcggtcaggaagtcagcgttaacaacttcgatgttcgggtgaccagacagtttttcacgcagagatttagccagacgcgggtcgatttcgtaagaggtaacctgacgagcacggtcagccagttcacgggtcagcagaccttcacccggaccagcttccagaaccggcaggtccggacgcagttcagcggtttcagcgatacgagcgatggttttacggtcacgcaggaagttctggccgaattggcggcggttacggtcacgctcggtacggccgaggacggggcgattctggttggggtgctggcggtcttggttgcggcggcgggggcggggctgttcatcggaggaggacatgacgatctcccgatgtgtcgtacgtatgggaattgacgaaaatcatatagattttcagttgaagtgtagcactgcatagtgtcatcgaagtgtcggcggcaacggtatgcccggtagggggtgggtctgcctttcggtttcgtgaacctgatgcggcgacgcgcatgtagccgataacccctagactcgcccgtgcagatcgtcggtgtggatccagatgtgtataagagacagctggtaccggccgctgct

SEQ ID NO: 14 - DNA, 9128 bp, synthetic construct
  source 1..9128: mol_type = other DNA
gtgcgtgcgggcgtgagcgtttctacgctgcggcgcaggaaatcagagcttgaggctgccggagcgacggtagacccgtccggttgggtggtgccactgcgtgcactcaaggtcgtttttggggtgtcagatgagacctcgaatgcgaataccagtaaatcctgacctgtgagttgtgaattcataggatagattctggaaactttaccgtccgagctccagcctgcggtccggcctgtcctgatcatgatccgtccgggggccgctagttgggcggtccccggacgattttgtgtacccgcagatgcgtgccagacaagcgcctcggctgttttgtgggtttgtgttggtggtgggggtgtgtgtagtgtgtgttgggccgttgggggctgcgtgtgtggttcttggtggtggctgtgtttgggatgtcgctgggacgcccgtagaactctgtgaggataaagtctcccttacagcctgcggtccggtaattttgtttaactttaagaaggagatatacatatgttcgtccaaatcgctgccagcctggcagccgcatcgtccattgcactcggcataccaggagctgccgagcaggaagtgccgatgaacctggtctcggctgatggcaaggaggtttccatcgggaagatcaccatccaggagaccccatacggtctgttgttcacccccgccctgcactcgctgagcgagggtattcacggtttccacgtccacgagaagggcaactgcgccccggcgcttaaagacggcaagccggtcgccgcgctgtccgccggtggtcactttgacccgaagaatactggcaagcacctgggcccgtggtcccctgacggccacctcggtgacctgccggccctgttcgtcacccatgacggcaaagccaactacccggtcctggccccgcgcctcaactccctgaaggagatcaagggccgctccctcatgctccacgctggtggcgacaatcaccacgaccacccagagcccctgggcggtggcggtgcccgcatggcctgcggcattatccagcatcatcaccatcaccactgataatcgctgggacgcccgctcgagcaataaacagttgatagggcttctccgttaccatggttcagccaaaaaacttaagaccgccggtcttgtccactaccttgcagtaatgcggtggacaggatcggcggttttcttttctcttctcaagctagcgaaatccctgaaactgagactgtagaaaataagcttccgaaactgaacctgttattttacgctacggacgcccggtcatgacgctgagttagtggcgcagctgcgctctgagaacgagtttttacggcgtcaggtcgagcagcaggcgcgcacgatcgaacggcaggctgaggcacacgcggtggtctcagcgcagctcacacgggttggccagcttgaggccggcgacgcagcagcaccgacactggcacccgttgaaaggccggctccgcgacggcggtggtggcagcgtcggtagcggtcaggatcgctctggcgtgacgagtgtgtctggcagtgcgaacagttgctcgaccagtggcagcagaagcgagatcgctgcgtggtgctgttcctcggtcagttcgtcgaggactggcgggtcttgctgcgtccagccgatcgcctcggcggccaaggtcagttccaagctgtgccaacgcacacgcccctcggctgacagctgagtctcgaactgtgcaactggaccggccggaagatgcacgttgccgaggtcgtgagtggccaagcgcacgtcaaagagtgctgcttcgtagccgcgcagaaatggcagtgctcggtcgattcggatcggcctgcccaggtacattccgggccgcttgatgaacgcctccgcgtagaagcgcaccgttctcggcccggcctcgtgatctgtcactgtgcacgctcctctcgatggttctcgacgctaccggagaccaccgacgttcatgcccagcgcagcgacctgaaaggaccaagccgagttagccgtgctaaccgtatagcttgctccgtcgcctctgagggcaaccacctgcgcagcaggtgggcggcagcccgcgcgcaagcgcctaccgggtttgggcacagcccataaatcaacgcctccggtgttgaagcgatcgtgtgtcacgattgctatgcttgctaccccttcagggttttcgtatacacaaatcaagttttttcgtatacgctaatgccatgagtgagcatctactgcacggcaagcccgtcaccaacgagcagattcaggcatgggcagacgaggccgaggccggatacgacctgcccaaactccccaagccacggcgcggacgcccgcccgtaggagacggtccgggcaccgtcgtacccgtgcgtctcgacgcggccaccgttgccgctctcacagaacgagcaacagccgagggcatcacgaaccgttcagacgcgatccgagccgcagtccacgagtggacacgggttgcctgacctccacgactcagcacgcaagcactaccaacgagaccggctcgacgacacggccgtgctctacgcggccacccacgttctcaactcccggccactcgacgacgaagacgacccgcgccgctggctcatgatcggaaccgacccagcaggccgcctactcgaactcgtcgcactgatctacgacgacggctacgaactgatcatccacgcaatgaaagcccgcacccaatacctcgaccagctctaaccaagaaaggaacctgatgagcgaccagctagacagcgaccgcaactacgacccgatgatcttcgacgtgatgcgcgagaccgcgaaccgcgtcgtcgccacgtacgttgcatgggaagatgaagccgctgatccccgcgaggctgcgcactggcaggccgagcgattccgcacccggcacgaggtgcgcgccgtcgaccctgacagccggcgagcagttcaggcgaagatcgcacagctgcgcgaggaactagccgcaatgcccgaacacgccccagccatcccttggagcaggtggcagcgtcaggggagtcgggggatgtttggcaggggatgtggaaagagagttcgctttgctcacatggctcaaccgggtaactaactgatatggggtcttcgtcgcccactttgaacacgccgaggaatggaccacgctgaacgtgactcgcatgcttcactgcatgtatggattcgttcgagacgttgttccctgagagctggctgccacgcaagccgctggcgtcagccgagaagtctggggcgtaccggcacgtgactcggcagagggcgctggagctgccttacatcgaagcgaacccgttggtcatgcagtccttggtcatcaccgatcgagatgcttcggatgctgactgggccgcagacctcgctgggctgccttcaccgtcctacgtgtccatgaaccgtgtcacgaccaccggacacatcgtctatgccttgaagaaccctgtgtgtctgaccgatgccgcgcggcgacggcctatcaacctgctcgcccgcgtcgagcagggcctatgcgacgttctcggcggcgatgcatcctacgggcaccggatcacaaagaacccgctcagcaccgcccatgcgaccctctggggccccgcagacgcgctctacgagctgcgcgccctcgcacacaccctcgacgagatccacgcactgccggaggcagggaacccgcgtcgcaacgtcacccgatcaacggtcggccgcaacgtcaccctgttcgacaccacccgcatgtgggcataccgggccgtccggcactcctggggcggcccggtcgccgaatgggagcacaccgtattcgagcacatccacctactgaacgagacgatcatcgccgacgaattcgccacaggccccctcggcttgaacgaacttaagcacttatctcgatccatttcccgatgggtctggcgcaacttcacccccgaaaccttccgcgcacgccagaaagcgatcagcctccgtggagcatccaaaggcggcaaagaaggcggccacaaaggcggcattgccagtggcgcatcacggcgcgcccatacccgtcaacagttcttggagggtctctcatgaccacacgtgaacgtctcccccgcaacggctacagcatcgccgctgctgcgaaaaagctcggtgtctccgagtccaccgtcaagcggtggacttccgagccacgcgaggagttcgtggcccgcgttgccgcacgccacgcgcggattcgtgagctgcgctcggagggtcagagcatgcgtgcgattgctgccgaggtcggggtttccgtgggcaccgtgcactacgcgctgaacaagaatcgaactgacgcatgaccgtaacgccgcacgatgagcattttcttgatcgtgcaccgcttggcactacgttcgcgtgcggttgcacagtgcgcgccacgttcttatcctgcggccattgtggctacagccaatggggggcatcagcaacggacgttgaacccggtgggcaagtgttactcagggggacatgcccagtctgcggcgctcggattgacggtatggcagtcgtgcatgcggccccaccgtcaaactcattcaggtatcagtgagaaccctcatggcaccccctcgtgacacgttctcgttgcgatcagctgcggccaagcttgatcttcgggcagcgttgggtcctggccacgggtgcgcatgatcgtgctcctgtcgttgaggacccggctaggctggcggggttgccttactggttagcagaatgaatcaccgatacgcgagcgaacgtgaagcgactgctgctgcaaaacgtctgcgacctgagcaacaacatgaatggtcttcggtttccgtgtttcgtaaagtctggaaacgcggaagtcagcgccctgcaccattatgttccggatctgcatcgcaggatgctgctggctaccctgtggaacacctacatctgtattaacgaagcgctggcattgaccctgagtgatttttctctggtcccgccgcatccataccgccagttgtttaccctcacaacgttccagtaaccgggcatgttcatcatcagtaacccgtatcgtgagcatcctctctcgtttcatcggtatcattacccccatgaacagaaatcccccttacacggaggcatcagtgaccaaacaggaaaaaaccgcccttaacatggcccgctttatcagaagccagacattaacgcttctggagaaactcaacgagctggacgcggatgaacaggcagacatctgtgaatcgcttcacgaccacgctgatgagctttaccgcagctgcctcgcgcgtttcggtgatgacggtgaaaacctctgacacatgcagctcccggagacggtcacagcttgtctgtaagcggatgccgggagcagacaagcccgtcagggcgcgtcagcgggtgttggcgggtgtcggggcgcagccatgacccagtcacgtagcgatagcggagtgtatactggcttaactatgcggcatcagagcagattgtactgagagtgcaccatatgcggtgtgaaataccgcacagatgcgtaaggagaaaataccgcatcaggcgctcttccgcttcctcgctcactgactcgctgcgctcggtcgttcggctgcggcgagcggtatcagctcactcaaaggcggtaatacggttatccacagaatcaggggataacgcaggaaagaacatgtgagcaaaaggccagcaaaaggccaggaaccgtaaaaaggccgcgttgctggcgtttttccataggctccgcccccctgacgagcatcacaaaaatcgacgctcaagtcagaggtggcgaaacccgacaggactataaagataccaggcgtttccccctggaagctccctcgtgcgctctcctgttccgaccctgccgcttaccggatacctgtccgcctttctcccttcgggaagcgtggcgctttctcatagctcacgctgtaggtatctcagttcggtgtaggtcgttcgctccaagctgggctgtgtgcacgaaccccccgttcagcccgaccgctgcgccttatccggtaactatcgtcttgagtccaacccggtaagacacgacttatcgccactggcagcagccactggtaacaggattagcagagcgaggtatgtaggcggtgctacagagttcttgaagtggtggcctaactacggctacactagaaggacagtatttggtatctgcgctctgctgaagccagttaccttcggaaaaagagttggtagctcttgatccggcaaacaaaccaccgctggtagcggtggtttttttgtttgcaagcagcagattacgcgcagaaaaaaaggatctcaagaagatcctttgatcttttctacggggtctgacgctcagtggaacgaaaactcacgttaagggattttggtcatgagattatcaaaaaggatcttcacctagatccttttaaattaaaaatgaagttttaaatcaatctaaagtatatatgagtaaacttggtctgacagttaccaatgcttaatcagtgaggcacctatctcagcgatctgtctatttcgttcatccatagttgcctgactccccgtcgtgtagataactacgatacgggagggcttaccatctggccccagtgctgcaatgataccgcgagacccacgctcaccggctccagatttatcagcaataaaccagccagccggaagggccgagcgcagaagtggtcctgcaactttatccgcctccatccagtctattaattgttgccgggaagctagagtaagtagttcgccagttaatagtttgcgcaacgttgttgccattgctgcaggcatcgtggtgtcacgctcgtcgtttggtatggcttcattcagctccggttcccaacgatcaaggcgagttacatgatcccccatgttgtgcaaaaaagcggttagctccttcggtcctccgatcgttgtcagaagtaagttggccgcagtgttatcactcatggttatggcagcactgcataattctcttactgtcatgccatccgtaagatgcttttctgtgactggtgagtactcaaccaagtcattctgagaatagtgtatgcggcgaccgagttgctcttgcccggcgtcaacacgggataataccgcgccacatagcagaactttaaaagtgctcatcattggaaaacgttcttcggggcgaaaactctcaaggatcttaccgctgttgagatccagttcgatgtaacccactcgtgcacccaactgatcttcagcatcttttactttcaccagcgtttctgggtgagcaaaaacaggaaggcaaaatgccgcaaaaaagggaataagggcgacacggaaatgttgaatactcatactcttcctttttcaatattattgaagcatttatcagggttattgtctcatgagcggatacatatttgaatgtatttagaaaaataaacaaataggggttccgcgcacatttccccgaaaagtgccacctgacgtctaagaaaccattattatcatgacattaacctataaaaataggcgtatcacgaggccctttcgtcttcaagaattcaagcttgtcgacgttaacctgcaggcatgcggatccggtaccagctgtctcttatacacatctctgcagttaacgctgacccggaccaccacgacgacccggacgaccaccggtacgaccaccaccagacggaccgcggcgaccaccctggtcaccctgttcacgttcaccggtacgaccgtcgtcacggttacgaccagaagaacgacggtcaccgtgaccagacgcttgccggtctctgcgatcttggcccccggtacgtctgtcaccacggtcctgaccaccggtacgacggtcgcccctatcctgtccacccgtcctacgaccacgctgcggctgaccaccacgcggttcgtttttctggtccagacgttcgaacagacgcagccactgttccggacgaacgtaagcaacaacagcaccaccaccaacaccagcgtggtccagagcagcttcaacacgacgacgcgggtatttacgcagcagagaagcctggatgttaccaccaacaccggtgaagcacagttcaaccatagattcgtaacgttccagagcagcaccttccagcagcggttcagcacgacgacgcagacgcatgatagcagagtcaactttcggaaccggtttgaacagacgacgatcgactttttcaacgaattcccattcgaacagcggccaggtcataacggtcagacgagaccaacgaccgtagtcaccggtacgtttacgagcgaattccagctgggtaaccatggtagcggtttcgatggtcggagcttccaggcaccagtcaacgatagcagaggtgataccgtacgggatagcaccaacgaaagcgaacggttccggcggcggttcagcggtcaggaagtcagcgttaacaacttcgatgttcgggtgaccagacagtttttcacgcagagatttagccagacgcgggtcgatttcgtaagaggtaacctgacgagcacggtcagccagttcacgggtcagcagaccttcacccggaccagcttccagaaccggcaggtccggacgcagttcagcggtttcagcgatacgagcgatggttttacggtcacgcaggaagttctggccgaattggcggcggttacggtcacgctcggtacggccgaggacggggcgattctggttggggtgctggcggtcttggttgcggcggcgggggcggggctgttcatcggaggaggacatgacgatctcccgatgtgtcgtacgtatgggaattgacgaaaatcatatagattttcagttgaagtgtagcactgcatagtgtcatcgaagtgtcggcggcaacggtatgcccggtagggggtgggtctgcctttcggtttcgtgaacctgatgcggcgacgcgcatgtagccgataacccctagactcgcccgtgcagatcgtcggtgtggatccagatgtgtataagagacagctggtaccggccgctgct

SEQ ID NO: 15 - DNA, 65 bp, synthetic construct
  source 1..65: mol_type = other DNA
cagcctgcggtccggttgacaccctatcagtgatagagtataatgctagctcgctgggacgcccg

SEQ ID NO: 16 - DNA, 2324 bp, synthetic construct
  source 1..2324: mol_type = other DNA
cagcctgcggtccggttgacaccctatcagtgatagagtataatgctagctcgctgggacgcccgtagaactctgtgaggataaagtctcccttacagcctgcggtccggtaattttgtttaactttaagaaggagatatacatatgttcgtccaaatcgctgccagcctggcagccgcatcgtccattgcactcggcataccaggagctgccgagcaggaagtgccgatgaacctggtctcggctgatggcaaggaggtttccatcgggaagatcaccatccaggagaccccatacggtctgttgttcacccccgccctgcactcgctgagcgagggtattcacggtttccacgtccacgagaagggcaactgcgccccggcgcttaaagacggcaagccggtcgccgcgctgtccgccggtggtcactttgacccgaagaatactggcaagcacctgggcccgtggtcccctgacggccacctcggtgacctgccggccctgttcgtcacccatgacggcaaagccaactacccggtcctggccccgcgcctcaactccctgaaggagatcaagggccgctccctcatgctccacgctggtggcgacaatcaccacgaccacccagagcccctgggcggtggcggtgcccgcatggcctgcggcattatccagcatcatcaccatcaccactgataatcgctgggacgcccgctcgagcaataaacagttgatagggcttctccgttaccatggttcagccaaaaaacttaagaccgccggtcttgtccactaccttgcagtaatgcggtggacaggatcggcggttttcttttctcttctcaattcttctgacctgtaacgaataatagatagtaaagtagtctccgattgagttttctctgccgagtcccacccagttctgtgatttcagtaagttggtaattgatacactgttgcgagaactggtgcctggtagtagataggttgttattgagtaagaaggtaaagtgaacgaaatccctgaaactgagactgtagaaaataagcttgtccagactattggatccaagagatttctacacgattgagcactgtctcctgcaggctcggtaccaaattccagaaaagaggcctcccgaaaggggggccttttttcgttttggtcctaatagataaaggataggtctggtagtgttgttcgttctcgcaggtaaatcaataatactctgcagttccgtagacttttcagtgggacagggtagcgataacagatagattgtaataagacacagtaggtgctcgtagttgcgtgaagagaaccgctcaggaaatccagtcagaagtattggtaatcgttgaaaactcagtcgaccagcctgcggtccggacaccgacgatctgcacgggcgagtctaggggttatcggctacatgcgcgtcgccgcatcaggttcacgaaaccgaaaggcagacccaccccctaccgggcataccgttgccgccgacacttcgatgacactatgcagtgctacacttcaactgaaaatctatatgattttcgtcaattctcgctgggacgcccgtagaactctgtgaggataaagtctcccttacagcctgcggtccggtaattttgtttaactttaagaaggagatatacatatgtcaagactagataagagcaaggtcattaacagcgcactggagttactaaacgaagttggaatagagggattgactacacgaaaattagcacagaaattaggagtagaacaaccgacactttattggcacgttaaaaataaaagagctttgctggatgctttagctatagaaatgctagaccgacaccacacacatttttgccccttagaaggagaaagttggcaagatttcctacgtaacaacgccaaatcatttagatgcgcgctattatcacaccgcgacggcgccaaagttcacctcgggacaagacctacggagaagcaatacgaaaccctagagaatcaattagcctttctatgtcaacaaggattcagtttggaaaacgccctctacgccctatcagccgttggtcattttacattgggatgcgttttagaggatcaggaacatcaagtagcaaaagaagaaagagagacacccaccaccgacagcatgccaccattattacgtcaagctattgaactattcgatcatcagggagcggaaccggcatttttatttggcctcgaattaatcatatgtggtttagaaaaacaattaaagtgtgaatctggatcccatcatcaccatcaccactgataatcgctgggacgcccg

SEQ ID NO: 17 - DNA, 7668 bp, synthetic construct
  source 1..7668: mol_type = other DNA
tctagaggaaatcagagcttgaggctgccggagcgacggtagacccgtccggttgggtggtgccactgcgtgcactcaaggtcgtttttggggtgtcagatgtgacctcgaatgcggaattcataggatagattctggaaactttaccgtccgagctccagcctgcggtccggttgacaccctatcagtgatagagtataatgctagctcgctgggacgcccgtagaactctgtgaggataaagtctcccttacagcctgcggtccggtaattttgtttaactttaagaaggagatatacatatgttcgtccaaatcgctgccagcctggcagccgcatcgtccattgcactcggcataccaggagctgccgagcaggaagtgccgatgaacctggtctcggctgatggcaaggaggtttccatcgggaagatcaccatccaggagaccccatacggtctgttgttcacccccgccctgcactcgctgagcgagggtattcacggtttccacgtccacgagaagggcaactgcgccccggcgcttaaagacggcaagccggtcgccgcgctgtccgccggtggtcactttgacccgaagaatactggcaagcacctgggcccgtggtcccctgacggccacctcggtgacctgccggccctgttcgtcacccatgacggcaaagccaactacccggtcctggccccgcgcctcaactccctgaaggagatcaagggccgctccctcatgctccacgctggtggcgacaatcaccacgaccacccagagcccctgggcggtggcggtgcccgcatggcctgcggcattatccagcatcatcaccatcaccactgataatcgctgggacgcccgctcgagcaataaacagttgatagggcttctccgttaccatggttcagccaaaaaacttaagaccgccggtcttgtccactaccttgcagtaatgcggtggacaggatcggcggttttcttttctcttctcaattcttctgacctgtaacgaataatagatagtaaagtagtctccgattgagttttctctgccgagtcccacccagttctgtgatttcagtaagttggtaattgatacactgttgcgagaactggtgcctggtagtagataggttgttattgagtaagaaggtaaagtgaacgaaatccctgaaactgagactgtagaaaataagcttgtccagactattggatccaagagatttctacacgattgagcactgtctcctgcaggctcggtaccaaattccagaaaagaggcctcccgaaaggggggccttttttcgttttggtcctaatagataaaggataggtctggtagtgttgttcgttctcgcaggtaaatcaataatactctgcagttccgtagacttttcagtgggacagggtagcgataacagatagattgtaataagacacagtaggtgctcgtagttgcgtgaagagaaccgctcaggaaatccagtcagaagtattggtaatcgttgaaaactcagtcgaccagcctgcggtccggacaccgacgatctgcacgggcgagtctaggggttatcggctacatgcgcgtcgccgcatcaggttcacgaaaccgaaaggcagacccaccccctaccgggcataccgttgccgccgacacttcgatgacactatgcagtgctacacttcaactgaaaatctatatgattttcgtcaattctcgctgggacgcccgtagaactctgtgaggataaagtctcccttacagcctgcggtccggtaattttgtttaactttaagaaggagatatacatatgtcaagactagataagagcaaggtcattaacagcgcactggagttactaaacgaagttggaatagagggattgactacacgaaaattagcacagaaattaggagtagaacaaccgacactttattggcacgttaaaaataaaagagctttgctggatgctttagctatagaaatgctagaccgacaccacacacatttttgccccttagaaggagaaagttggcaagatttcctacgtaacaacgccaaatcatttagatgcgcgctattatcacaccgcgacggcgccaaagttcacctcgggacaagacctacggagaagcaatacgaaaccctagagaatcaattagcctttctatgtcaacaaggattcagtttggaaaacgccctctacgccctatcagccgttggtcattttacattgggatgcgttttagaggatcaggaacatcaagtagcaaaagaagaaagagagacacccaccaccgacagcatgccaccattattacgtcaagctattgaactattcgatcatcagggagcggaaccggcatttttatttggcctcgaattaatcatatgtggtttagaaaaacaattaaagtgtgaatctggatcccatcatcaccatcaccactgataatcgctgggacgcccggacgtcctattacactcgtcgttggaaactgaagatgcggccgcggaaacacagaaaaaagcccgcacctgacagtgcgggctttttttttcgaccaaaggtagcgaacgacgagtcactgttgaggataaatactttctctactagctagctgttacacaggtcctcagcggcgcgcccgcccggtcatgacgctgagttagtggcgcagctgcgctctgagaacgagtttcgaccctgacagccggcgagctgttcaggcgaagatcgcacagctgcgcgaggaactagccgcaatgcccgaacacgccccagccatcccttggagcaggtggcagcgtcaggggagtcgggggatgtttggcaggggatgtggaaagagagttcgctttgctcacatggctcaaccgggtaactaactgatatgggctcttcgtcgcccactttgaacacgccgaggaatggaccacgctgaacgtgactcgcatgcttcactgcatgtatggattcgttcgagactttgttccctgagagctggctgccacgcaagccgctggcgtcagccgagaagtctggggcgtaccggcacgtgactcggcagagggcgctggagctgccttacatcgaagcgaacccgttggtcatgcagtccttggtcatcaccgatcgagatgcttcggatgctgactgggccgcagacctcgctgggctgccttcaccgtcctacgtgtccatgaaccgtgtcacgaccaccggacacatcgtctatgccttgaagaaccctgtgtgtctgaccgatgccgcgcggcgacggcctatcaacctgctcgcccgcgtcgagcagggcctatgcgacgttctcggcggcgatgcatcctacgggcaccggatcacaaagaacccgctcagcaccgcccatgcgaccctctggggccccgcagacgcgctctacgagctgcgcgccctcgcacacaccctcgacgagatccacgcactgccggaggcagggaacccgcgtcgcaacgtcacccgatcaacggtcggccgcaacgtcaccctgttcgacaccacccgcatgtgggcataccgggccgtccggcactcctggggcggcccggtcgccgaatgggagcacaccgtattcgagcacatccacctactgaacgaaacgatcatcgccgacgagttcgccacaggccccctcggcttgaacgaacttaagcacttatctcgatccatttcccgatgggtctggcgcaacttcacccccgaaaccttccgcgcacgccagaaagcgatcagcctccgtggagcatccaaaggcggcaaagaaggcggccacaaaggcggcattgccagtggcgcatcacggcgtgcccatacccgtcaacagttcttggagggtctgtcatgaccacacgtgaacgcctcccccgcaacggctacagcatcgccgccgctgcgaaaaagctcggtgtctccgagtccaccgtcaagcggtggacttccgagccacgcgaggagttcgtggcccgcgttgccgcacgccacgcgcggattcgtgagctgcgctcggagggtcagagcatgcgtgcgattgctgccgaggtcggggtttccgtgggcaccgtgcactacgcgctgaacaagaatcgaactgacgcatgaccgtaacgccgcacgatgagcattttcttgatcgtgcaccgcttggcactacgttcgcgtgcggttgcacagtgcgcgccacgttcttatcctgcggccattgtggctacagccaatggggggcatcagcaacggacgttgaacccggtgggcaagtgttactcagggggacatgcccagtctgcggcgctcggattgacggtatggcagtcgtgcatgcggccccaccgtcaaactcattcaggtatcagtgagaaccctcatggcaccccctcgtgacacgttctcgttgcgatcagctgcggccaagctgatcttcgggcagcgttgggtcctggccacgggtgcgcatgatcgtgctcctgtcgttgaggacccggctaggctggcggggttgccttactgatcaggccgcgttgctggcgtttttccataggctccgcccccctgacgagcatcacaaaaatcgacgctcaagtcagaggtggcgaaacccgacaggactataaagataccaggcgtttccccctggaagctccctcgtgcgctctcctgttccgaccctgccgcttaccggatacctgtccgcctttctcccttcgggaagcgtggcgctttctcatagctcacgctgtaggtatctcagttcggtgtaggtcgttcgctccaagctgggctgtgtgcacgaaccccccgttcagcccgaccgctgcgccttatccggtaactatcgtcttgagtccaacccggtaagacacgacttatcgccactggcagcagccactggtaacaggattagcagagcgaggtatgtaggcggtgctacagagttcttgaagtggtggcctaactacggctacactagaaggacagtatttggtatctgcgctctgctgaagccagttaccttcggaaaaagagttggtagctcttgatccggcaaacaaaccaccgctggtagcggtggtttttttgtttgcaagcagcagattacgcgcagaaaaaaaggatctcaagaagatcctttgatcttttctacggggtctgacgctcagtggaacgaaaactcacgttaagggattttggtcatgaggcgcctcaccaatgcttgatgagggaggcaccgatctcggcgatctgacggttgcgctcatccatcgtggcctgggagccggtcgtgtagatcaccacgatgcggctgggcttaccgtcgggaccgagagccgcgatgatgccacgcgagccgcgctcaccagcacccgacttgtccgcgatgaaccaaccggccgggagcgcgctgcgcaacagcgggccagcgaccttgtcggcctccatccagtcgatcagttgctgacgggaggccagagtgaggagttcaccggtcaggagtttacggagggtggtagccatagccgcgggcatagtcgtgtcgcgctcgtcgttcgggatagcctcattaagttcgggttcccaacggtccagacgggtcacgtggtcgcccatgttgtggagaaaagccgtcagctctttcgggccaccgatggtcgtcaacagcagattggcggcagtgttgtcggacatagtgatggccgcggagcacagctcgcgcacggtcatcccatcggtcagatgtttctccgtgaccggggagtattcgaccaggtcgttctgggagtaatgaatgcgacggcccagttgctcctgcccagcatccacccggctaagcacagcgccgcagaggaggaccttgaacgtggacatcatggggaaacgctcctcagggcggaaagactccagaatcttaccggagttcaggtccaactcgatataaccgacgcgcgcccccagctgatcctcggcgtccttgaccttgaccagggtttccggatgggcaaaaaccggcaagcaaaaggccgcaaaaaatgggataagggcaacgcggaagtgctggatcgacatactcttcctttttcaatattattgaagcatttatcagggttattgtctcatgagcggatacatatttgaatgtatttagaaaaataaacaaataggggttccgcgactagttccccgaaaagtgccacctgacgttaagaaaccattattatcatgacattaacctataaaaataggcgtatcacgaggccctttcgtctacaatcagcgctgacccggaccgccacgacggcctggacgaccgccggtacgaccaccacccgaagggccacgacgaccaccctggtcgccctgctcgcgctccccggtacgaccatcgtcgcgattacggccagaggaccgacggtcaccgtggccggaggcctgacggtcgcgacggtcctgaccacccgtccgacggtcgccacgatcctggccacccgtacggcggtcaccacgatcctgaccacccgtacgacggccgcgctgcggttggccaccgcgcggctcgttcttctggtcaaggcgctcgaagagccgcagccattgctccggccggacgtaggccacgacagcaccaccacccacgccggcatggtccagcgcagcctccacgcgacgacgagggtacttgcgcaggagggaggcttgaatgttgccgccgacaccagtaaaacacaactccaccatgctctcgtagcgctcaagggcagcaccctccaacagcggttcagcgcggcgacgcagacgcatgatggcggaatcgaccttcgggaccggcttgaacaagcggcgatcgaccttctcgacgaactcccactcgaagagcggccaagtcatgaccgtgaggcgggaccagcggccataatcaccggtgcgcttacgggcaaattcgagttgggtaaccatcgtggcggtttcgatcgtcggagcctccaggcaccaatcgacgatcgcagacgtgatgccgtacgggatcgcgccgacgaaggcaaacggctcgggagggggctcggcggtcaggaagtccgcgttgacgacctcgatattcgggtggccggacagcttctcacgcagggacttcgccaagcgcgggtcgatctcgtagctcgtcacctggcgggcccgatcggcaagctcacgggtcagcagaccctcgcctgggccagcctccaggaccggaaggtcggggcgcagttcggccgtttccgcgatgcgggcgatcgtcttacggtcacgaaggaaattctgaccgaattgacggcggttgcggtcccgctcagtacggcccaggaccgggcggttctggttcgggtgctggcggtcctggttgcggcgacgcgggcgcggttgctcgtcggacgacgacatgacgatctcccgatgtgtcgtacgtatgggaattgacgaaaatcatatagattttcagttgaagtgtagcactgcatagtgtcatcgaagtgtcggcggcaacggtatgcccggtagggggtgggtctgcctttcggtttcgtgaacctgatgcggcgacgcgcatgtagccgataacccctagactcgcccgtgcagatcgtcggtgt

SEQ ID NO: 18 - DNA, 462 bp, synthetic construct
  source 1..462: mol_type = other DNA
atggtgaggcgcagcaggaatctatccgacgctgttgatcttgcggtgatcgacaaggacgctgccatcttcgccatctcagtggcggcagagctcgccggaatgcaccctcagaccctgcgcacttacgatcggctcgggcttgtagtgcccgaacgcactcgggggcgggggcgtcgctactcgatgcgtgacgttgctgcgttgcggatggtccagcatctgtcccaggaagaggggattaacctcaacggcatccgaaggatccttcagatggaacgtaggatcgaacagttgtcggagcaggtggacgagctcaccgacaccgtgcgtgggatgcaagtggcgcgttaccagggcagtgaagatccgagagtctttactgctgagtcgaccggccgggtgcatatgggtcggacggtcgttcatgcccagttggcactgccttctcatcgtggttga

SEQ ID NO: 19 - DNA, 250 bp, synthetic construct
  source 1..250: mol_type = other DNA
cgtgaagtgcggaagctgccggacggttcgccgtccggcatttttcatggtcggaaggggtcgtctgaggatgtcttgacgagactttcggtgggtgggaatactcccgccggatcgtcggttgagtgtagcgaactcaacttcatgaaaaatcagccaacgtcaacttgagtgctcgtgactcagggtctagagttgagtcgaagtcgctcaaggggatgtagtcccagaacattcgtccatcaggagg

SEQ ID NO: 20 - DNA, 112 bp, synthetic construct
  source 1..112: mol_type = other DNA
ggttaaggccgcccaatacatctacacccacccaggcgaggtgtgccccgccaagtgggaagaaggcgatgagaccctcgccccgtcgatcgacctcgtcggcaagatctga

SEQ ID NO: 21 - DNA, 140 bp, synthetic construct
  source 1..140: mol_type = other DNA
gaccatgggggcatcatgccacgggtgcgggccctggcgacacagagagtcccgagttcatgatctttatagctattgactatagatgctggtttagtgatagccttgatctatcacatcgtcgacgagaaaggacaccc

SEQ ID NO: 22 - DNA, 945 bp, synthetic construct
  source 1..945: mol_type = other DNA
gtgaaccttcatgatctgcggtatttcgtcgccctggccgaagaacaccacttcggccgggctgcggcgtcatgcggtgtcagccagcccaccctctcaactcaaatccaccggctcgagaacgagctcggcgtggtgctggccgtgagggtgggacgacgcatcgagatcaccccagtgggggaacgcatcgcccaagctgcccgtgacatgttggtgctatccgacgacatccggaccatggcgcgggaggaagccgaccggatgaccctccagctgagggtcggggtattccccaccttagggccgttcgtgttgcctcaggtgatcgcccgatgtgaccagcacgagcctggcgtgaacatccatatcgtcgagaagcgcacggcagagctgttggaggcaatccgcaacggacagttagacgtcgccgcagtggcagcccccgttaatgatgactctttggtgactattcccgtttttcgggaggagttcttgctcgtgacgggggctgacgatgagttggcccgtgaggaacgaccaatcaatccgcacgacgttcccaccgaagggctcatcctcatgtcggagggacactgtctaagagaccaggtgcttgaggtgtgcagcccgtctcatccgctgcctcccgacaccctcacggcgggatccctcgagacgctccgcgaactcgtatcggtgggcgccggtcaaaccctcatgccgcgcagtgcgatctcggcaccacttcatgcggacccgcgcatcgtggtgcgggagttcacccaccccagaccccaccgcgacatcgtggtggctggcagaccggccacaatgcaccgtccggcggtgcagaccctgaccaccatcctgcggcagctaccaggtgacgtcgtcgagcctctcggcgttgccggagcatcgttgtgctctcacgggatgtga

SEQ ID NO: 23 - DNA, 15 bp, unidentified
  source 1..15: mol_type = other DNA
cagcctgcggtccgg

SEQ ID NO: 24 - DNA, 15 bp, synthetic construct
  source 1..15: mol_type = other DNA
tcgctgggacgcccg